European Patent Application EP 4 272 739 A1, published November 8, 2023. Title: Composition for inhibiting cancer metastasis and enhancing sensitivity to anticancer agent. Applicant: Korea Advanced Institute of Science and Technology. The sequence listing filed with the application follows.

SEQUENCE LISTING (31 sequences)

SEQ ID NO: 1 - RNA, 21 nt, Artificial Sequence
  shS4
taccatacagagaacattgga

SEQ ID NO: 2 - RNA, 21 nt, Artificial Sequence
  shERK1
cctgaattgtatcatcaacat

SEQ ID NO: 3 - RNA, 21 nt, Artificial Sequence
  shERK2
ccatgaggcaagaaactatat

SEQ ID NO: 4 - DNA, 23 bp, Artificial Sequence
  SMAD4 forward primer
cagcctcccatttccaatcatcc

SEQ ID NO: 5 - DNA, 22 bp, Artificial Sequence
  SMAD4 reverse primer
gatctcctccagaagggtccac

SEQ ID NO: 6 - DNA, 20 bp, Artificial Sequence
  GRHL2 forward primer
gtgccttaggcctgttggat

SEQ ID NO: 7 - DNA, 20 bp, Artificial Sequence
  GRHL2 reverse primer
ttctcttgaagggggaacgc

SEQ ID NO: 8 - DNA, 22 bp, Artificial Sequence
  OVOL2 forward primer
catgcccaaagtcttcctggtg

SEQ ID NO: 9 - DNA, 21 bp, Artificial Sequence
  OVOL2 reverse primer
actgggatgtaggtgtctgcc

SEQ ID NO: 10 - DNA, 21 bp, Artificial Sequence
  NCAD forward primer
gtcagctgtcggtgacaaagc

SEQ ID NO: 11 - DNA, 24 bp, Artificial Sequence
  NCAD reverse primer
gatcaagtccagctgccactgtga

SEQ ID NO: 12 - DNA, 20 bp, Artificial Sequence
  FN1 forward primer
cttctggtcagcaacccagt

SEQ ID NO: 13 - DNA, 20 bp, Artificial Sequence
  FN1 reverse primer
accgtgtgggtacaggtgat

SEQ ID NO: 14 - DNA, 22 bp, Artificial Sequence
  ZEB1 forward primer
agcagtgaaagagaagggaatg

SEQ ID NO: 15 - DNA, 22 bp, Artificial Sequence
  ZEB1 reverse primer
tgacagcagtgtcttgttgttg

SEQ ID NO: 16 - DNA, 21 bp, Artificial Sequence
  MYC forward primer
gtcaagaggcgaacacacaac

SEQ ID NO: 17 - DNA, 21 bp, Artificial Sequence
  MYC reverse primer
ttggacggacaggatgtatgc

SEQ ID NO: 18 - DNA, 27 bp, Artificial Sequence
  ECAD forward primer
gaagattgcaccggtcgacaaaggaca

SEQ ID NO: 19 - DNA, 27 bp, Artificial Sequence
  ECAD reverse primer
gcagctgatgggaggaataacccagtc

SEQ ID NO: 20 - DNA, 21 bp, Artificial Sequence
  TWIST forward primer
tcggacaagctgagcaagatt

SEQ ID NO: 21 - DNA, 20 bp, Artificial Sequence
  TWIST reverse primer
gcagcttgccatcttggagt

SEQ ID NO: 22 - DNA, 18 bp, Artificial Sequence
  SNAI1 forward primer
gctgctacaaggccatgt

SEQ ID NO: 23 - DNA, 18 bp, Artificial Sequence
  SNAI1 reverse primer
cggactcttggtgcttgt

SEQ ID NO: 24 - DNA, 22 bp, Artificial Sequence
  CD90 forward primer
gaaggtcctctacttatccgcc

SEQ ID NO: 25 - DNA, 22 bp, Artificial Sequence
  CD90 reverse primer
tgatgccctcacacttgaccag

SEQ ID NO: 26 - DNA, 18 bp, Artificial Sequence
  VIM forward primer
ccaggcaaagcaggagtc

SEQ ID NO: 27 - DNA, 18 bp, Artificial Sequence
  VIM reverse primer
cgaaggtgacgagccatt

SEQ ID NO: 28 - DNA, 20 bp, Artificial Sequence
  b-Actin forward primer
agagctacgagctgcctgac

SEQ ID NO: 29 - DNA, 20 bp, Artificial Sequence
  b-Actin reverse primer
agcactgtgttggcgtacag

SEQ ID NO: 30 - DNA, 25 bp, Artificial Sequence
  GAPDH forward primer
tgatgacatcaagaaggtggtgaag

SEQ ID NO: 31 - DNA, 23 bp, Artificial Sequence
  GAPDH reverse primer
tccttggaggccatgtgggccat